European Patent Application EP 4 606 898 A1, published August 27, 2025. Title: Surface-display overexpression technique by using lipoprotein PrsA expression system. Applicant: Future and Tech co. Application KR. The sequence listing filed with the application follows.

SEQUENCE LISTING (17 sequences)

SEQ ID NO: 1 - DNA, 912 bp, Lactobacillus sakei
  source 1..912: mol_type = genomic DNA
atgatgaaaaaatggctattagccgctgccagtctattaatggtagttacattagcaggttgtggaagcaacactatcgcaactcttaagggtggtaaagtcactcaagacgaattctacaaagaaattaaggaaacttctgccggcaagcaacaagtacaacaaatgatcttgcaaaaagcacttcaagaacaatatggtagcaagagtcttactaagaaaatcgacaagacttacaatacttacaagaaacaatacggttcatctttcacttcagtacttgcacaaagtggtttaacaacctcttcattcaaaaaccaaatcacaactcaaatgttagctaacgctgctttaaaagctaacaaaaaagttacaaacgctgatttgaagaaacaatggaaaacatacgaaccaaaagttgaagtacaacatatcttagttgaaaagaaagatactgctgaaacagttatttctgaacttaagaaagacaactcaactaaaaacttcactgctttagctaagaagtactcaacagatactggtactaagaaagacggcggtaaattacctgtctttgatagcacagatacatcattagatccaacattcaaaacagctgccttcaagttgaagacaaacgaatacacaacaacacctgttaagacatcatatggttaccacgttatccgcatgatcaagaaccctggtaaaggtaagatggctgatcacaagaagacattaactgaccaagtttatgctaagtgggctaatgatcaaacagtgatggctaaggtttacacgaaggttcttaagaaagccgacgtaacaatcaaggataaagatttatcagatatcctttcaagctacggcgttaacgctaaaaaatcatcagctaaatcatcatcaaaataa

SEQ ID NO: 2 - protein, 303 aa, Lactobacillus sakei
MMKKWLLAAASLLMVVTLAGCGSNTIATLKGGKVTQDEFYKEIKETSAGKQQVQQMILQKALQEQYGSKSLTKKIDKTYNTYKKQYGSSFTSVLAQSGLTTSSFKNQITTQMLANAALKANKKVTNADLKKQWKTYEPKVEVQHILVEKKDTAETVISELKKDNSTKNFTALAKKYSTDTGTKKDGGKLPVFDSTDTSLDPTFKTAAFKLKTNEYTTTPVKTSYGYHVIRMIKNPGKGKMADHKKTLTDQVYAKWANDQTVMAKVYTKVLKKADVTIKDKDLSDILSSYGVNAKKSSAKSSSK

SEQ ID NO: 3 - DNA, 300 bp, Lactobacillus sakei
  source 1..300: mol_type = genomic DNA
gaaatcaaaacaacagctgttgattcactcgctgatatcagcgatgctgttcaaactttttcgtttgaagctcaaccccgggttgcacaaatttcagaatcaatcaaacgtcttacggacgatttaaaggcgctataacgcagtttatcaacctttcacggacgtattcataaaaaagctaaatttgaaggttctgtgaaattttcgctctcggatttaattcagcgggttcatgtgttatattaattgatgaattcacggtattaatcgtatttacaataatttataaggatgtgtcat

SEQ ID NO: 4 - protein, 23 aa, Lactobacillus sakei
DLSDILSSYGVNAKKSSAKSSSK

SEQ ID NO: 5 - protein, 5 aa, Lactobacillus sakei
KDNST

SEQ ID NO: 6 - protein, 10 aa, Lactobacillus sakei
WANDQTVMAK

SEQ ID NO: 7 - DNA, 28 bp, synthetic construct
  source 1..28: mol_type = other DNA
aaactgcaggaaatcaaaacaacagctg

SEQ ID NO: 8 - DNA, 39 bp, synthetic construct
  source 1..39: mol_type = other DNA
ttttctatattattaggatccttttgatgatgatttgac

SEQ ID NO: 9 - DNA, 26 bp, synthetic construct
  source 1..26: mol_type = other DNA
aaaaggatccatgagcaaaggagaag

SEQ ID NO: 10 - DNA, 27 bp, synthetic construct
  source 1..27: mol_type = other DNA
tcttggtacctttgtagagctcatcca

SEQ ID NO: 11 - DNA, 46 bp, synthetic construct
  source 1..46: mol_type = other DNA
ggggggtaccttatcaggatcctttatccttgattgttacgtcggc

SEQ ID NO: 12 - DNA, 28 bp, synthetic construct
  source 1..28: mol_type = other DNA
ccccctcgagaagaagtactcaacagat

SEQ ID NO: 13 - DNA, 28 bp, synthetic construct
  source 1..28: mol_type = other DNA
ccccctcgagcttaagttcagaaataac

SEQ ID NO: 14 - DNA, 28 bp, synthetic construct
  source 1..28: mol_type = other DNA
ccccctcgagaagaagtactcaacagat

SEQ ID NO: 15 - DNA, 28 bp, synthetic construct
  source 1..28: mol_type = other DNA
ccccctcgagcttaagttcagaaataac

SEQ ID NO: 16 - DNA, 27 bp, synthetic construct
  source 1..27: mol_type = other DNA
aaaggatccgacttgtacgtggtggag

SEQ ID NO: 17 - DNA, 48 bp, synthetic construct
  source 1..48: mol_type = other DNA
gggtctagaactagtgtcgacttagttgattttgcggtatggggcatt